European Patent Specification EP 3 635 398 B1, published July 24, 2024. Title: CHIMERIC RECEPTOR FOR USE IN WHOLE-CELL SENSORS FOR DETECTING ANALYTES OF INTEREST. Applicant: Inserm. The sequence listing filed with the application follows.

SEQUENCE LISTING (18 sequences)

SEQ ID NO: 1 - protein, 151 aa, Artificial Sequence
  CadC transcriptional activator
MQQPVVRVGEWLVTPSINQISRNGRQLTLEPRLIDLLVFFAQHSGEVLSRDELIDNVWKRSIVTNHVVTQSISELRKSLKDNDEDSPVYIATVPKRGYKLMVPVIWYSEEEGEEIMLSSPPPIPEAVPATDSPSHSLNIQNTATPPEQSPV

SEQ ID NO: 2 - protein, 155 aa, Artificial Sequence
  CadC transcriptional activator DNA binding domain
MQQPVVRVGEWLVTPSINQISRNGRQLTLEPRLIDLLVFFAQHSGEVLSRDELIDNVWKRSIVTNHVVTQSISELRKSLKDNDEDSPVYIATVPKRGYKLMVPVIWYSEEEGEEIMLSSPPPIPEAVPATDSPSHSLNIQNTATPPEQSPVKSKR

SEQ ID NO: 3 - protein, 24 aa, Artificial Sequence
  transmembrane domain
GGPGLLLLLLLLLLLLLLLLGPGG

SEQ ID NO: 4 - protein, 26 aa, Artificial Sequence
  transmembrane domain
FTTFWVWFFFLLSLGICVALVAFSSL

SEQ ID NO: 5 - protein, 24 aa, Artificial Sequence
  transmembrane domain
ITLIIFGVMAAGVIGTILLISYGI

SEQ ID NO: 6 - protein, 24 aa, Artificial Sequence
  transmembrane domain
LLLILLGVLALGVLLTLLLLLLLL

SEQ ID NO: 7 - protein, 7 aa, Artificial Sequence
  spacer
DTRLPMS

SEQ ID NO: 8 - protein, 186 aa, Artificial Sequence
  chimeric recpetor domain
MQQPVVRVGEWLVTPSINQISRNGRQLTLEPRLIDLLVFFAQHSGEVLSRDELIDNVWKRSIVTNHVVTQSISELRKSLKDNDEDSPVYIATVPKRGYKLMVPVIWYSEEEGEEIMLSSPPPIPEAVPATDSPSHSLNIQNTATPPEQSPVKSKRGGPGLLLLLLLLLLLLLLLLGPGGDTRLPMS

SEQ ID NO: 9 - DNA, 162 bp, Artificial Sequence
  promoter
atccattgtaaacattaaatgtttatcttttcatgatatcaacttgcgatcctgatgtgttaataaaaaacctcaagttctcacttacagaaacttttgtgttatttcacctaatctttaggattaatccttttttcgtgagtaatcttatcgccagtttgg

SEQ ID NO: 10 - protein, 33 aa, Artificial Sequence
  wtTM (CadC156-188)
FTTFWVWFFFLLSLGICVALVAFSSLDTRLPMS

SEQ ID NO: 11 - protein, 24 aa, Artificial Sequence
  artTM
GGPGLLLLLLLLLLLLLLLLGPGG

SEQ ID NO: 12 - protein, 5 aa, Artificial Sequence
  SEQ ID NO:12
GGGSG

SEQ ID NO: 13 - protein, 87 aa, Artificial Sequence
  SEQ ID NO:13
MKALTARQQEVFDLIRDHISQTGMPPTRAEIAQRLGFRSASSAEEHLKALARKGVIEIVSGASRGIRLLQEEEEGLPLVGRVAAGEP

SEQ ID NO: 14 - protein, 5 aa, Artificial Sequence
  SEQ ID NO:14
QEEEE

SEQ ID NO: 15 - DNA, 80 bp, Artificial Sequence
  SEQ ID NO:15
cgaggctctttccgaaaatagggttgatctttgttgtcactggatgtacctacatccatacggtaactcacaggggctgg

SEQ ID NO: 16 - protein, 7 aa, Artificial Sequence
  SEQ ID NO:16
DTRLPMS

SEQ ID NO: 17 - protein, 5 aa, Artificial Sequence
  SEQ ID NO:17
GGGSG

SEQ ID NO: 18 - protein, 5 aa, Artificial Sequence
  SEQ ID NO:18
EAAAK